European Patent Application EP 4 488 384 A1, published January 8, 2025. Title: PRIMERS FOR SELECTIVE AMPLIFICATION OF RARE TARGET SEQUENCES. Applicant: Infiniplex Ltd. The sequence listing filed with the application follows.

SEQUENCE LISTING (43 sequences)

SEQ ID NO: 1 - DNA, 195 bp, synthetic construct
  source 1..195: mol_type = other DNA
tttattataaggcctgctgaaaatgactgaatataaacttgtggtagttggagctgatggcgtaggcaagagtgccttgacgatacagctaattcagaatcattttgtggacgaatatgatccaacaatagaggtaaatcttgttttaatatgcatattactggtgcaggaccattctttgatacagataaaggt

SEQ ID NO: 2 - DNA, 249 bp, synthetic construct
  source 1..249: mol_type = other DNA
ctgtttcgtatttatagctgatttgatggagttggacatggccatggaaccagacagaaaagcggctgttagtcactggcagcaacagtcttacctggactctggaatccattctggtgccactgccacagctccttctctgagtggtaaaggcaatcctgaggaagaggatgtggatacctcccaagtcctgtatgagtgggaacagggattttctcagtccttcactcaagaacaagtagctggtaa

SEQ ID NO: 3 - DNA, 248 bp, synthetic construct
  source 1..248: mol_type = other DNA
agggtcttctctgtttcagggcatgaactacttggaggaccgtcgcttggtgcaccgcgacctggcagccaggaacgtactggtgaaaacaccgcagcatgtcaagatcacagattttgggatggccaaactgctgggtgcggaagagaaagaataccatgcagaaggaggcaaagtaaggaggtggctttaggtcagccagcattttcctgacaccagggaccaggctgccttcccactagctgtat

SEQ ID NO: 4 - DNA, 238 bp, synthetic construct
  source 1..238: mol_type = other DNA
tcctgagtattggtgttccattgcttactttgaaatggatgttcaggtaggagagacatttaaggttccttcaagctgccctattgttactgttgatggatacgtggacccttctggaggagatcacttttgtttgggtcaactctccaatgtccacaggacagaagccattgagagagcaaggtattgattgtatagtcagatagttactttaaaaaattgagcatagtacattgtc

SEQ ID NO: 5 - DNA, 195 bp, synthetic construct
  source 1..195: mol_type = other DNA
tttattataaggcctgctgaaaatgactgaatataaacttgtggtagttggagctggtggcgtaggcaagagtgccttgacgatacagctaattcagaatcattttgtggacgaatatgatccaacaatagaggtaaatcttgttttaatatgcatattactggtgcaggaccattctttgatacagataaaggt

SEQ ID NO: 6 - DNA, 248 bp, synthetic construct
  source 1..248: mol_type = other DNA
agggtcttctctgtttcagggcatgaactacttggaggaccgtcgcttggtgcaccgcgacctggcagccaggaacgtactggtgaaaacaccgcagcatgtcaagatcacagattttgggctggccaaactgctgggtgcggaagagaaagaataccatgcagaaggaggcaaagtaaggaggtggctttaggtcagccagcattttcctgacaccagggaccaggctgccttcccactagctgtat

SEQ ID NO: 7 - DNA, 249 bp, synthetic construct
  source 1..249: mol_type = other DNA
ctgtttcgtatttatagctgatttgatggagttggacatggccatggaaccagacagaaaagcggctgttagtcactggcagcaacagtcttacctggactctggaatccattctggtgccacagccacagctccttctctgagtggtaaaggcaatcctgaggaagaggatgtggatacctcccaagtcctgtatgagtgggaacagggattttctcagtccttcactcaagaacaagtagctggtaa

SEQ ID NO: 8 - DNA, 238 bp, synthetic construct
  source 1..238: mol_type = other DNA
tcctgagtattggtgttccattgcttactttgaaatggatgttcaggtaggagagacatttaaggttccttcaagctgccctattgttactgttgatggatacgtggacccttctggaggagatcgcttttgtttgggtcaactctccaatgtccacaggacagaagccattgagagagcaaggtattgattgtatagtcagatagttactttaaaaaattgagcatagtacattgtc

SEQ ID NO: 9 - DNA, 66 bp, synthetic construct
  source 1..66: mol_type = other DNA
tttattataaggcctgctgaaaatgactgaatataaacttgtggtagttggcagctattaagctga

SEQ ID NO: 10 - DNA, 56 bp, synthetic construct
  source 1..56: mol_type = other DNA
gcctgctgaaaatgactgaatataaacttgtggtagttgcagatcattagagctga

SEQ ID NO: 11 - DNA, 68 bp, synthetic construct
  source 1..68: mol_type = other DNA
tttattataaggcctgctgaaaatgactgaatataaacttgtggtagtactgcaccattaggagctga

SEQ ID NO: 12 - DNA, 57 bp, synthetic construct
  source 1..57: mol_type = other DNA
tttattataaggcctgctgaaaatgactgaatataaacctgcaccattaggagctga

SEQ ID NO: 13 - DNA, 44 bp, synthetic construct
  source 1..44: mol_type = other DNA
acctggactctggaatccattctggtagtggcatatagccactg

SEQ ID NO: 14 - DNA, 48 bp, synthetic construct
  source 1..48: mol_type = other DNA
caacagtcttacctggactctggaatccatagtggcatatagccactg

SEQ ID NO: 15 - DNA, 47 bp, synthetic construct
  source 1..47: mol_type = other DNA
cagcaacagtcttacctggactctggaatagtggcatatagccactg

SEQ ID NO: 16 - DNA, 48 bp, synthetic construct; identical to SEQ ID NO: 14
  source 1..48: mol_type = other DNA

SEQ ID NO: 17 - DNA, 35 bp, synthetic construct
  source 1..35: mol_type = other DNA
caccgcagcatgtcaagatcacacccattttggga

SEQ ID NO: 18 - DNA, 36 bp, synthetic construct
  source 1..36: mol_type = other DNA
ggtgaaaacaccgcagcatgtcaacccattttggga

SEQ ID NO: 19 - DNA, 41 bp, synthetic construct
  source 1..41: mol_type = other DNA
gtactggtgaaaacaccgcagcatgacccaacttcttggga

SEQ ID NO: 20 - DNA, 43 bp, synthetic construct
  source 1..43: mol_type = other DNA
accgcagcatgtcaagatcacagacccaaaacttcttttggga

SEQ ID NO: 21 - DNA, 45 bp, synthetic construct
  source 1..45: mol_type = other DNA
ggtgaaaacaccgcagcatgtcaacccaaaatcttcattttggga

SEQ ID NO: 22 - DNA, 46 bp, synthetic construct
  source 1..46: mol_type = other DNA
caccgcagcatgtcaagatcacacccaaaatcattagattttggga

SEQ ID NO: 23 - DNA, 22 bp, synthetic construct
  source 1..22: mol_type = other DNA
gatcatattcgtccacaaaatg

SEQ ID NO: 24 - DNA, 25 bp, synthetic construct
  source 1..25: mol_type = other DNA
gggaggtatccacatcctcttcctc

SEQ ID NO: 25 - DNA, 22 bp, synthetic construct
  source 1..22: mol_type = other DNA
gcctccttctgcatggtattct

SEQ ID NO: 26 - DNA, 27 bp, synthetic construct
  source 1..27: mol_type = other DNA
gactgaatataaacttgtggtagttgg

SEQ ID NO: 27 - DNA, 28 bp, synthetic construct
  source 1..28: mol_type = other DNA
tcttacctggactctggaatccattctg

SEQ ID NO: 28 - DNA, 18 bp, synthetic construct
  source 1..18: mol_type = other DNA
ctggcagccaggaacgta

SEQ ID NO: 29 - DNA, 88 bp, synthetic construct
  source 1..88: mol_type = other DNA
acgtgccctcaatacgagcccccttcaccaacggcctgctgaaaatgactgaatataaacacacagtctgagcccactctggagctga

SEQ ID NO: 30 - DNA, 47 bp, synthetic construct
  source 1..47: mol_type = other DNA
cagcaacagtcttacctggactctggagcgagtaataagagccactg

SEQ ID NO: 31 - DNA, 47 bp, synthetic construct
  source 1..47: mol_type = other DNA
actggtgaaaacaccgcagcatgttgcacgagtgagccattttggga

SEQ ID NO: 32 - DNA, 47 bp, synthetic construct
  source 1..47: mol_type = other DNA
agctgccctattgttactgttgatggaagatctccattaggagatca

SEQ ID NO: 33 - DNA, 48 bp, synthetic construct
  misc_feature 47: note = RNA
  source 1..48: mol_type = other DNA
agctgccctattgttactgttgatggaagatctccattaggagatrca

SEQ ID NO: 34 - DNA, 47 bp, synthetic construct; identical to SEQ ID NO: 32
  misc_feature 27: note = RNA
  source 1..47: mol_type = other DNA

SEQ ID NO: 35 - DNA, 48 bp, synthetic construct
  misc_feature 47: note = RNA
  source 1..48: mol_type = other DNA
agctgccctattgttactgttgatggraagatctccattaggagatca

SEQ ID NO: 36 - DNA, 20 bp, synthetic construct
  source 1..20: mol_type = other DNA
tccttcaagctgccctattg

SEQ ID NO: 37 - DNA, 24 bp, synthetic construct
  source 1..24: mol_type = other DNA
ctctctcaatggcttctgtcctgt

SEQ ID NO: 38 - DNA, 73 bp, synthetic construct
  source 1..73: mol_type = other DNA
gaagaaaagtgttttgaaatgtgttttataatttagactagtgaatatttccgtgttcctattaaggaacacc

SEQ ID NO: 39 - DNA, 70 bp, synthetic construct
  source 1..70: mol_type = other DNA
gaagaaaagtgttttgaaatgtgttttataatttagactagtgaatatttgcgtgttcattagaacaccg

SEQ ID NO: 40 - DNA, 249 bp, synthetic construct
  source 1..249: mol_type = other DNA
tttttagatattcccattattatagagatgattgttgaattttccttttggggaagaaaagtgttttgaaatgtgttttataatttagactagtgaatatttttctttgttttttaaggaacaccgtccattggcatggggaaatataaacttgtttgattacacagacactctagtatctggaaaaatggctttgaatctttggccagtacctcatggattagaagatttgctgaaccctattggtgt

SEQ ID NO: 41 - DNA, 249 bp, synthetic construct
  source 1..249: mol_type = other DNA
tttttagatattcccattattatagagatgattgttgaattttccttttggggaagaaaagtgttttgaaatgtgttttataatttagactagtgaatatttttctttgttttttaaggaacactgtccattggcatggggaaatataaacttgtttgattacacagacactctagtatctggaaaaatggctttgaatctttggccagtacctcatggattagaagatttgctgaaccctattggtgt

SEQ ID NO: 42 - DNA, 26 bp, synthetic construct
  source 1..26: mol_type = other DNA
ccatgaggtactggccaaagattcaa

SEQ ID NO: 43 - DNA, 48 bp, synthetic construct
  source 1..48: mol_type = other DNA
ggaagaaaagtgttttgaaatgtgttttataatttagactagtgaata